European Patent Application EP 4 435 091 A1, published September 25, 2024. Title: NOVEL STREPTOCOCCUS SALIVARIUS STRAIN HAVING ANTIBACTERIAL, ANTIFUNGAL, ANTIINFLAMMATORY ACTIVITY AND INHIBITING DENTAL CARIES AND ORAL COMPOSITION COMPRISING THE SAME. Applicant: 그린스토어. Application EP, filed June 23, 2023. The sequence listing filed with the application follows.

SEQUENCE LISTING (13 sequences)

SEQ ID NO: 1 - RNA, 1470 nt, Streptococcus salivarius
  source 1..1470: mol_type = rRNA
gacgaacgctggcggcgtgcctaatacatgcaagtagaacgctgaagagaggagcttgctcttcttggatgagttgcgaacgggtgagtaacgcgtaggtaacctgccttgtagcgggggataactattggaaacgatagctaataccgcataacaatggatgacccatgtcatttatttgaaaggggcaaatgctccactacaagatggacctgcgttgtattagctagtaggtgaggtaacggctcacctaggcgacgatacatagccgacctgagagggtgatcggccacactgggactgagacacggcccagactcctacgggaggcagcagtagggaatcttcggcaatgggggcaaccctgaccgagcaacgccgcgtgagtgaagaaggttttcggatcgtaaagctctgttgtaagtcaagaacgagtgtgagagtggaaagttcacactgtgacggtagcttaccagaaagggacggctaactacgtgccagcagccgcggtaatacgtaggtcccgagcgttgtccggatttattgggcgtaaagcgagcgcaggcggtttgataagtctgaagttaaaggctgtggctcaaccatagttcgctttggaaactgtcaaacttgagtgcagaaggggagagtggaattccatgtgtagcggtgaaatgcgtagatatatggaggaacaccggtggcgaaagcggctctctggtctgtaactgacgctgaggctcgaaagcgtggggagcgaacaggattagataccctggtagtccacgccgtaaacgatgagtgctaggtgttggatcctttccgggattcagtgccgcagctaacgcattaagcactccgcctggggagtacgaccgcaaggttgaaactcaaaggaattgacgggggcccgcacaagcggtggagcatgtggtttaattcgaagcaacgcgaagaaccttaccaggtcttgacatcccgatgctatttctagagatagaaagttacttcggtacatcggtgacaggtggtgcatggttgtcgtcagctcgtgtcgtgagatgttgggttaagtcccgcaacgagcgcaacccctattgttagttgccatcattcagttgggcactctagcgagactgccggtaataaaccggaggaaggtggggatgacgtcaaatcatcatgccccttatgacctgggctacacacgtgctacaatggttggtacaacgagttgcgagtcggtgacggcaagctaatctcttaaagccaatctcagttcggattgtaggctgcaactcgcctacatgaagtcggaatcgctagtaatcgcggatcagcacgccgcggtgaatacgttcccgggccttgtacacaccgcccgtcacaccacgagagtttgtaacacccgaagtcggtgaggtaaccttttggagccagccgcctaaggtgggatagatgattggggtg

SEQ ID NO: 2 - DNA, 20 bp, synthetic construct
  source 1..20: mol_type = other DNA
gtgaaggtgcagttttgcca

SEQ ID NO: 3 - DNA, 19 bp, synthetic construct
  source 1..19: mol_type = other DNA
tctccacaaccctctgcac

SEQ ID NO: 4 - DNA, 20 bp, synthetic construct
  source 1..20: mol_type = other DNA
cagggacctctctctaatca

SEQ ID NO: 5 - DNA, 20 bp, synthetic construct
  source 1..20: mol_type = other DNA
agctggttatctctcagctc

SEQ ID NO: 6 - DNA, 18 bp, synthetic construct
  source 1..18: mol_type = other DNA
gtggtggacctgacctgc

SEQ ID NO: 7 - DNA, 20 bp, synthetic construct
  source 1..20: mol_type = other DNA
tgagcttgacaaagtggtcg

SEQ ID NO: 8 - DNA, 20 bp, synthetic construct
  source 1..20: mol_type = other DNA
aagcaacgcgaagaacctta

SEQ ID NO: 9 - DNA, 20 bp, synthetic construct
  source 1..20: mol_type = other DNA
gtctcgctagagtgcccaac

SEQ ID NO: 10 - DNA, 20 bp, synthetic construct
  source 1..20: mol_type = other DNA
ctacactttcgggtggcttg

SEQ ID NO: 11 - DNA, 24 bp, synthetic construct
  source 1..24: mol_type = other DNA
gaagcttttcaccattagaagctg

SEQ ID NO: 12 - DNA, 21 bp, synthetic construct
  source 1..21: mol_type = other DNA
ttgccacatcttcactcgctt

SEQ ID NO: 13 - DNA, 22 bp, synthetic construct
  source 1..22: mol_type = other DNA
gtttagtagcaacttctggctt